European Patent Application EP 4 400 515 A2, published July 17, 2024. Title: Enzyme and pathway modulation with sulfhydryl compounds and their derivatives. Applicant: F. Hoffmann-La Roche AG. Application EP. The sequence listing filed with the application follows.

SEQUENCE LISTING (47 sequences)

SEQ ID NO: 1 - DNA, 1047 bp, synthetic construct
  source 1..1047: mol_type = other DNA; note = The cDNA sequence of UDP-glucose 4-epimerase in CHO K1M
  CDS 1..1047: note = /transl_table=1
atggccgagaaggtgctggtcacaggcggagctggctacattggcagccacacggtactggagctgctggaggcaggctacgcccctgtggtcatcgacaacttccataatgccattcgtggaggggattccatgcctgagagcctgcggcgggtccaggaactgacaggccgctctgtggagtttgaggagatggacatcttggaccaggcagcgctacagcacctctttaagaagcacagctttaaggctgtcatccactttgctgggctcaaggctgtgggcgagtcggtgcagaagcctctggattattatagagttaacctaacagggaccatccagcttctggagatcatgagggcccacggggtgaagaatctcgtgttcagcagctcagccaccgtgtatgggaatccccagtacctgcctctggatgaggcccaccccaccgggggttgtaccaacccctatggaaagtccaagttcttcatcgaggagatggtccgggacctgtgccgggcagattcggcctggaacgcagtgctgctacgctacttcaatcccacgggtgcccacgcctctggccgcatcggcgaggatccccagggcgtccccaacaacctcatgccctatgtctcccaggtggcaattgggcgacgagaggccctgaatgtctttggtggtgactatgatacagaggatggcacaggtgtaagggattacattcatgtggtggatctggcgaagggccacatcgcagccttgaagaagctgaaggagcaatgtggttgccggatctacaacctgggcacaggcacaggctactctgtcctgcagatggtccaagcaatggagaaggcttcagggaagaagatcccatacaaggtggtggcacggcgggaaggtgacgtggcagcctgttatgccaaccccagcctggcccatgaggagctgggctggacagcagccttggggctggacaggatgtgtgaagatctatggcgctggcagaagcagaacccttcaggctttggagcacaggcctaa

SEQ ID NO: 2 - protein, 348 aa, synthetic construct
  source 1..348: note = [CDS]:1..1047 from SEQ ID NO 1
MAEKVLVTGGAGYIGSHTVLELLEAGYAPVVIDNFHNAIRGGDSMPESLRRVQELTGRSVEFEEMDILDQAALQHLFKKHSFKAVIHFAGLKAVGESVQKPLDYYRVNLTGTIQLLEIMRAHGVKNLVFSSSATVYGNPQYLPLDEAHPTGGCTNPYGKSKFFIEEMVRDLCRADSAWNAVLLRYFNPTGAHASGRIGEDPQGVPNNLMPYVSQVAIGRREALNVFGGDYDTEDGTGVRDYIHVVDLAKGHIAALKKLKEQCGCRIYNLGTGTGYSVLQMVQAMEKASGKKIPYKVVARREGDVAACYANPSLAHEELGWTAALGLDRMCEDLWRWQKQNPSGFGAQA

SEQ ID NO: 3 - DNA, 1140 bp, synthetic construct
  source 1..1140: mol_type = other DNA; note = The cDNA sequence of UDP-alpha-D-glucose: alpha-D-galactose-1-phosphate uridylyltransferase in CHO K1M
  CDS 1..1140: note = /transl_table=1
atgtcgcaaaacggagatgatcctgagcagcgccagcaggcgtcagaggcggacgccatggcagcgaccttccgggcgagcgaacaccagcatattcgctacaatccgctccaggatgagtgggtgttagtgtcggcccatcgcatgaagcggccctggcaaggacaagtggagccccagcttctgaagacagtgccccgctatgacccactcaaccctctgtgtcccggggccacacgagccaatggggaggtgaatccacactatgacagcaccttcctgtttgacaatgacttcccagctctgcagcccgatgctccggatccaggacccagtgaccatcctctttttcgagcagaggcggccagaggagtttgtaaggtcatgtgcttccatccctggtcggatgtgacactgccactcatgtcagtccctgagatccgagctgtcatcgatgcctgggcttcagtcaccgaggatctgggtgcccagtatccttgggtgcagatctttgaaaacaaaggagccatgatgggctgttctaacccccacccccactgccaggtttgggccagcagtttcctgccagatattgcccagcgtgaagtgcgatcccagcagaactatcacagccagcatggagaacctctgttactggaatatggccgccaagaactcctcaggaaggaacgtctggtcttatctagtgagcactggctagtcctggttcccttctgggcagtgtgggctttccagacactactgctgccccgccggcatgtacgtcggctacctgagctgacccctgctgaacgtgatgatctagcctccatcatgaagaagctattgaccaagtatgacaacctatttgagacatcttttccctactccatgggctggcatggggctcccacgggattaaagactggagccgcctatgaccactggcagctacatgctcattactatcccccactcctgcgctctgctactgtccggaaattcatggttggctatgaaatgcttgcccatgggcaccgggacctcactcctgaacaggctgcagagagactaagggcgcttcctgaggtacattattgcctggcaaagaaagacaaggaaacagcagctgttgcttga

SEQ ID NO: 4 - protein, 379 aa, synthetic construct
  source 1..379: note = [CDS]:1..1140 from SEQ ID NO 3
MSQNGDDPEQRQQASEADAMAATFRASEHQHIRYNPLQDEWVLVSAHRMKRPWQGQVEPQLLKTVPRYDPLNPLCPGATRANGEVNPHYDSTFLFDNDFPALQPDAPDPGPSDHPLFRAEAARGVCKVMCFHPWSDVTLPLMSVPEIRAVIDAWASVTEDLGAQYPWVQIFENKGAMMGCSNPHPHCQVWASSFLPDIAQREVRSQQNYHSQHGEPLLLEYGRQELLRKERLVLSSEHWLVLVPFWAVWAFQTLLLPRRHVRRLPELTPAERDDLASIMKKLLTKYDNLFETSFPYSMGWHGAPTGLKTGAAYDHWQLHAHYYPPLLRSATVRKFMVGYEMLAHGHRDLTPEQAAERLRALPEVHYCLAKKDKETAAVA

SEQ ID NO: 5 - DNA, 21 bp, synthetic construct
  source 1..21: mol_type = other DNA; note = forward primer UDP_GlcE-F2-21
atggccgagaaggtgctggtc

SEQ ID NO: 6 - DNA, 21 bp, synthetic construct
  source 1..21: mol_type = other DNA; note = reverse primer UDP_GlcE-R21
ttaggcctgtgctccaaagcc

SEQ ID NO: 7 - DNA, 21 bp, synthetic construct
  source 1..21: mol_type = other DNA; note = forward primer UDP-Gal-T-F2-21
atgtcgcaaaacggagatgat

SEQ ID NO: 8 - DNA, 18 bp, synthetic construct
  source 1..18: mol_type = other DNA; note = reverse primer UDP-Gal-T-R18
tcaagcaacagctgctgt

SEQ ID NO: 9 - protein, 140 aa, synthetic construct
  source 1..140: note = Synthesized
MDVFMKGLSKAKEGVVAAAEKTKQGVAEAAGKTKEGVLYVGSKTKEGVVHGVATVAEKTKEQVTNVGGAVVTGVTAVAQKTVEGAGSIAAATGFVKKDQLGKNEEGAPQEGILEDMPVDPDNEAYEMPSEEGYQDYEPEA

SEQ ID NO: 10 - protein, 5 aa, synthetic construct
  source 1..5: note = alpha-synuclein; CDR1 of heavy chain (CDR-H1)
NYGMS

SEQ ID NO: 11 - protein, 17 aa, synthetic construct
  source 1..17: note = alpha-synuclein; CDR2 of heavy chain (CDR-H2)
SISSGGGSTYYPDNVKG

SEQ ID NO: 12 - protein, 7 aa, synthetic construct
  source 1..7: note = alpha-synuclein; CDR3 of heavy chain (CDR-H3)
GGAGIDY

SEQ ID NO: 13 - protein, 17 aa, synthetic construct
  source 1..17: note = alpha-synuclein; CDR1 of light chain (CDR-L1)
KSIQTLLYSSNQKNYLA

SEQ ID NO: 14 - protein, 7 aa, synthetic construct
  source 1..7: note = alpha-synuclein; CDR2 of light chain (CDR-L2)
WASIRKS

SEQ ID NO: 15 - protein, 9 aa, synthetic construct
  source 1..9: note = alpha-synuclein; CDR3 of light chain (CDR-L3)
QQYYSYPLT

SEQ ID NO: 16 - protein, 116 aa, synthetic construct
  source 1..116: note = alpha-synuclein; heavy chain variable domain (VH)
EVQLVESGGGLVQPGGSLRLSCAASGFTFSNYGMSWVRQAPGKGLEWVASISSGGGSTYYPDNVKGRFTISRDDAKNSLYLQMNSLRAEDTAVYYCARGGAGIDYWGQGTLVTVSS

SEQ ID NO: 17 - protein, 113 aa, synthetic construct
  source 1..113: note = alpha-synuclein; light chain variable domain (VL)
DIQMTQSPSSLSASVGDRVTITCKSIQTLLYSSNQKNYLAWFQQKPGKAPKLLIYWASIRKSGVPSRFSGSGSGTDFTLTISSLQPEDLATYYCQQYYSYPLTFGGGTKLEIK

SEQ ID NO: 18 - protein, 328 aa, synthetic construct
  source 1..328: note = alpha-synuclein; heavy chain constant domain (CH)
ASTKGPSVFPLAPSSKSTSGGTAALGCLVKDYFPEPVTVSWNSGALTSGVHTFPAVLQSSGLYSLSSVVTVPSSSLGTQTYICNVNHKPSNTKVDKRVEPKSCDKTHTCPPCPAPELLGGPSVFLFPPKPKDTLMISRTPEVTCVVVDVSHEDPEVKFNWYVDGVEVHNAKTKPREEQYNSTYRVVSVLTVLHQDWLNGKEYKCKVSNKALPAPIEKTISKAKGQPREPQVYTLPPSREEMTKNQVSLTCLVKGFYPSDIAVEWESNGQPENNYKTTPPVLDSDGSFFLYSKLTVDKSRWQQGNVFSCSVMHEALHNHYTQKSLSLSP

SEQ ID NO: 19 - protein, 107 aa, synthetic construct [sequence omitted]

SEQ ID NO: 20 - protein, 444 aa, synthetic construct
  source 1..444: note = alpha-synuclein; heavy chain (H)
EVQLVESGGGLVQPGGSLRLSCAASGFTFSNYGMSWVRQAPGKGLEWVASISSGGGSTYYPDNVKGRFTISRDDAKNSLYLQMNSLRAEDTAVYYCARGGAGIDYWGQGTLVTVSSASTKGPSVFPLAPSSKSTSGGTAALGCLVKDYFPEPVTVSWNSGALTSGVHTFPAVLQSSGLYSLSSVVTVPSSSLGTQTYICNVNHKPSNTKVDKRVEPKSCDKTHTCPPCPAPELLGGPSVFLFPPKPKDTLMISRTPEVTCVVVDVSHEDPEVKFNWYVDGVEVHNAKTKPREEQYNSTYRVVSVLTVLHQDWLNGKEYKCKVSNKALPAPIEKTISKAKGQPREPQVYTLPPSREEMTKNQVSLTCLVKGFYPSDIAVEWESNGQPENNYKTTPPVLDSDGSFFLYSKLTVDKSRWQQGNVFSCSVMHEALHNHYTQKSLSLSP

SEQ ID NO: 21 - protein, 220 aa, synthetic construct
  source 1..220: note = alpha-synuclein; light chain (L)
DIQMTQSPSSLSASVGDRVTITCKSIQTLLYSSNQKNYLAWFQQKPGKAPKLLIYWASIRKSGVPSRFSGSGSGTDFTLTISSLQPEDLATYYCQQYYSYPLTFGGGTKLEIKRTVAAPSVFIFPPSDEQLKSGTASVVCLLNNFYPREAKVQWKVDNALQSGNSQESVTEQDSKDSTYSLSSTLTLSKADYEKHKVYACEVTHQGLSSPVTKSFNRGEC

SEQ ID NO: 22 - protein, 5 aa, synthetic construct
  source 1..5: note = CD3; CDR1 of heavy chain (CDR-H1)
TYAMN

SEQ ID NO: 23 - protein, 19 aa, synthetic construct
  source 1..19: note = CD3; CDR2 of heavy chain (CDR-H2)
RIRSKYNNYATYYADSVKG

SEQ ID NO: 24 - protein, 14 aa, synthetic construct
  source 1..14: note = CD3; CDR3 of heavy chain (CDR-H3)
HGNFGNSYVSWFAY

SEQ ID NO: 25 - protein, 14 aa, synthetic construct
  source 1..14: note = CD3; CDR1 of light chain (CDR-L1)
GSSTGAVTTSNYAN

SEQ ID NO: 26 - protein, 7 aa, synthetic construct
  source 1..7: note = CD3; CDR2 of light chain (CDR-L2)
GTNKRAP

SEQ ID NO: 27 - protein, 9 aa, synthetic construct
  source 1..9: note = CD3; CDR3 of light chain (CDR-L3)
ALWYSNLWV

SEQ ID NO: 28 - protein, 125 aa, synthetic construct
  source 1..125: note = CD3; heavy chain variable domain (VH)
EVQLLESGGGLVQPGGSLRLSCAASGFTFSTYAMNWVRQAPGKGLEWVSRIRSKYNNYATYYADSVKGRFTISRDDSKNTLYLQMNSLRAEDTAVYYCVRHGNFGNSYVSWFAYWGQGTLVTVSS

SEQ ID NO: 29 - protein, 109 aa, synthetic construct
  source 1..109: note = CD3; light chain variable domain (VL)
QAVVTQEPSLTVSPGGTVTLTCGSSTGAVTTSNYANWVQEKPGQAFRGLIGGTNKRAPGTPARFSGSLLGGKAALTLSGAQPEDEAEYYCALWYSNLWVFGGGTKLTVL

SEQ ID NO: 30 - protein, 101 aa, synthetic construct
  source 1..101: note = CD3; heavy chain constant domain (CH)
ASTKGPSVFPLAPSSKSTSGGTAALGCLVKDYFPEPVTVSWNSGALTSGVHTFPAVLQSSGLYSLSSVVTVPSSSLGTQTYICNVNHKPSNTKVDKKVEPK

SEQ ID NO: 31 - protein, 107 aa, synthetic construct
  source 1..107: note = CD3; light chain constant domain (CL)
ASVAAPSVFIFPPSDEQLKSGTASVVCLLNNFYPREAKVQWKVDNALQSGNSQESVTEQDSKDSTYSLSSTLTLSKADYEKHKVYACEVTHQGLSSPVTKSFNRGEC

SEQ ID NO: 32 - protein, 101 aa, synthetic construct; identical to SEQ ID NO: 30
  source 1..101: note = CD3 heavy chain constant domain (CD3 CH)

SEQ ID NO: 33 - protein, 232 aa, synthetic construct
  source 1..232: note = CD3; light chain (L)
EVQLLESGGGLVQPGGSLRLSCAASGFTFSTYAMNWVRQAPGKGLEWVSRIRSKYNNYATYYADSVKGRFTISRDDSKNTLYLQMNSLRAEDTAVYYCVRHGNFGNSYVSWFAYWGQGTLVTVSSASVAAPSVFIFPPSDEQLKSGTASVVCLLNNFYPREAKVQWKVDNALQSGNSQESVTEQDSKDSTYSLSSTLTLSKADYEKHKVYACEVTHQGLSSPVTKSFNRGEC

SEQ ID NO: 34 - protein, 5 aa, synthetic construct
  source 1..5: note = CD20; CDR1 of heavy chain (CDR-H1)
YSWIN

SEQ ID NO: 35 - protein, 17 aa, synthetic construct
  source 1..17: note = CD20; CDR2 of heavy chain (CDR-H2)
RIFPGDGDTDYNGKFKG

SEQ ID NO: 36 - protein, 10 aa, synthetic construct
  source 1..10: note = CD20; CDR3 of heavy chain (CDR-H3)
NVFDGYWLVY

SEQ ID NO: 37 - protein, 16 aa, synthetic construct
  source 1..16: note = CD20; CDR1 of light chain (CDR-L1)
RSSKSLLHSNGITYLY

SEQ ID NO: 38 - protein, 7 aa, synthetic construct
  source 1..7: note = CD20; CDR2 of light chain (CDR-L2)
QMSNLVS

SEQ ID NO: 39 - protein, 9 aa, synthetic construct
  source 1..9: note = CD20; CDR3 of light chain (CDR-L3)
AQNLELPYT

SEQ ID NO: 40 - protein, 119 aa, synthetic construct
  source 1..119: note = CD20; heavy chain variable domain (VH)
QVQLVQSGAEVKKPGSSVKVSCKASGYAFSYSWINWVRQAPGQGLEWMGRIFPGDGDTDYNGKFKGRVTITADKSTSTAYMELSSLRSEDTAVYYCARNVFDGYWLVYWGQGTLVTVSS

SEQ ID NO: 41 - protein, 115 aa, synthetic construct
  source 1..115: note = CD20; light chain variable domain (VL)
DIVMTQTPLSLPVTPGEPASISCRSSKSLLHSNGITYLYWYLQKPGQSPQLLIYQMSNLVSGVPDRFSGSGSGTDFTLKISRVEAEDVGVYYCAQNLELPYTFGGGTKVEIKRTV

SEQ ID NO: 42 - protein, 101 aa, synthetic construct
  source 1..101: note = CD20; heavy chain constant domain (CH)
ASTKGPSVFPLAPSSKSTSGGTAALGCLVEDYFPEPVTVSWNSGALTSGVHTFPAVLQSSGLYSLSSVVTVPSSSLGTQTYICNVNHKPSNTKVDEKVEPK

SEQ ID NO: 43 - protein, 104 aa, synthetic construct
  source 1..104: note = CD20; light chain constant domain (CL)
AAPSVFIFPPSDRKLKSGTASVVCLLNNFYPREAKVQWKVDNALQSGNSQESVTEQDSKDSTYSLSSTLTLSKADYEKHKVYACEVTHQGLSSPVTKSFNRGEC

SEQ ID NO: 44 - protein, 219 aa, synthetic construct
  source 1..219: note = CD20 light chain (CD20 VL-CL)
DIVMTQTPLSLPVTPGEPASISCRSSKSLLHSNGITYLYWYLQKPGQSPQLLIYQMSNLVSGVPDRFSGSGSGTDFTLKISRVEAEDVGVYYCAQNLELPYTFGGGTKVEIKRTVAAPSVFIFPPSDRKLKSGTASVVCLLNNFYPREAKVQWKVDNALQSGNSQESVTEQDSKDSTYSLSSTLTLSKADYEKHKVYACEVTHQGLSSPVTKSFNRGEC

SEQ ID NO: 45 - protein, 447 aa, synthetic construct
  source 1..447: note = CD20 heavy chain [CD20 VH-CHl(EE)-Fc (hole, P329G LALA)]
QVQLVQSGAEVKKPGSSVKVSCKASGYAFSYSWINWVRQAPGQGLEWMGRIFPGDGDTDYNGKFKGRVTITADKSTSTAYMELSSLRSEDTAVYYCARNVFDGYWLVYWGQGTLVTVSSASTKGPSVFPLAPSSKSTSGGTAALGCLVEDYFPEPVTVSWNSGALTSGVHTFPAVLQSSGLYSLSSVVTVPSSSLGTQTYICNVNHKPSNTKVDEKVEPKSCDKTHTCPPCPAPEAAGGPSVFLFPPKPKDTLMISRTPEVTCVVVDVSHEDPEVKFNWYVDGVEVHNAKTKPREEQYNSTYRVVSVLTVLHQDWLNGKEYKCKVSNKALGAPIEKTISKAKGQPREPQVCTLPPSRDELTKNQVSLSCAVKGFYPSDIAVEWESNGQPENNYKTTPPVLDSDGSFFLVSKLTVDKSRWQQGNVFSCSVMHEALHNHYTQKSLSLSP

SEQ ID NO: 46 - protein, 439 aa, synthetic construct
  source 1..439: note = CD20-CD3 heavy chain [CD3 VL-CH1-Fc (knob, P329G LALA)]
QAVVTQEPSLTVSPGGTVTLTCGSSTGAVTTSNYANWVQEKPGQAFRGLIGGTNKRAPGTPARFSGSLLGGKAALTLSGAQPEDEAEYYCALWYSNLWVFGGGTKLTVLSSASTKGPSVFPLAPSSKSTSGGTAALGCLVKDYFPEPVTVSWNSGALTSGVHTFPAVLQSSGLYSLSSVVTVPSSSLGTQTYICNVNHKPSNTKVDKKVEPKSCDKTHTCPPCPAPEAAGGPSVFLFPPKPKDTLMISRTPEVTCVVVDVSHEDPEVKFNWYVDGVEVHNAKTKPREEQYNSTYRVVSVLTVLHQDWLNGKEYKCKVSNKALGAPIEKTISKAKGQPREPQVYTLPPCRDELTKNQVSLWCLVKGFYPSDIAVEWESNGQPENNYKTTPPVLDSDGSFFLYSKLTVDKSRWQQGNVFSCSVMHEALHNHYTQKSLSLSP

SEQ ID NO: 47 - protein, 673 aa, synthetic construct
  source 1..673: note = CD20 heavy chain [CD20 VH-CHl(EE)-CD3 VL-CH1-Fc (knob, P329G LALA)]
QVQLVQSGAEVKKPGSSVKVSCKASGYAFSYSWINWVRQAPGQGLEWMGRIFPGDGDTDYNGKFKGRVTITADKSTSTAYMELSSLRSEDTAVYYCARNVFDGYWLVYWGQGTLVTVSSASTKGPSVFPLAPSSKSTSGGTAALGCLVEDYFPEPVTVSWNSGALTSGVHTFPAVLQSSGLYSLSSVVTVPSSSLGTQTYICNVNHKPSNTKVDEKVEPKSCDGGGGGSGGGGSQAVVTQEPSLTVSPGGTVTLTCGSSTGAVTTSNYANWVQEKPGQAFRGLIGGTNKRAPGTPARFSGSLLGGKAALTLSGAQPEDEAEYYCALWYSNLWVFGGGTKLTVLSSASTKGPSVFPLAPSSKSTSGGTAALGCLVKDYFPEPVTVSWNSGALTSGVHTFPAVLQSSGLYSLSSVVTVPSSSLGTQTYICNVNHKPSNTKVDKKVEPKSCDKTHTCPPCPAPEAAGGPSVFLFPPKPKDTLMISRTPEVTCVVVDVSHEDPEVKFNWYVDGVEVHNAKTKPREEQYNSTYRVVSVLTVLHQDWLNGKEYKCKVSNKALGAPIEKTISKAKGQPREPQVYTLPPCRDELTKNQVSLWCLVKGFYPSDIAVEWESNGQPENNYKTTPPVLDSDGSFFLYSKLTVDKSRWQQGNVFSCSVMHEALHNHYTQKSLSLSP